European Patent Application EP 4 722 247 A1, published April 8, 2026. Title: 靶向CD39的抗原结合蛋白及其应用. Applicant: 原启生物科技（上海）有限责任公司. The sequence listing filed with the application follows.

SEQUENCE LISTING (71 sequences)

SEQ ID NO: 1 - protein, 8 aa, synthetic construct
  REGION 1..8: note = B391-F04/B391-hF04 HCDR1
GFTFSNLG

SEQ ID NO: 2 - protein, 8 aa, synthetic construct
  REGION 1..8: note = B391-F04/B391-hF04 HCDR2
ISASGDYT

SEQ ID NO: 3 - protein, 8 aa, synthetic construct
  REGION 1..8: note = B391-F04/B391-hF04 HCDR3
TRRVDSYP

SEQ ID NO: 4 - protein, 25 aa, synthetic construct
  REGION 1..25: note = B391-F04/B393-D07/B39C6-G06 H-FR1
QLQLVESGGGLVQPGGSLRLSCAAS

SEQ ID NO: 5 - protein, 17 aa, synthetic construct
  REGION 1..17: note = B391-F04/B391-hF04 H-FR2
MSWYRQAPGKAREWVGS

SEQ ID NO: 6 - protein, 38 aa, synthetic construct
  REGION 1..38: note = B391-F04 H-FR3
TYQNSVKGRFTISRDNAKNTLYLQMNNLKPEDTGVYYC

SEQ ID NO: 7 - protein, 11 aa, synthetic construct
  REGION 1..11: note = B391-F04 H-FR4
RGQGTQVTVSS

SEQ ID NO: 8 - protein, 115 aa, synthetic construct
  REGION 1..115: note = B391-F04 VHH
QLQLVESGGGLVQPGGSLRLSCAASGFTFSNLGMSWYRQAPGKAREWVGSISASGDYTTYQNSVKGRFTISRDNAKNTLYLQMNNLKPEDTGVYYCTRRVDSYPRGQGTQVTVSS

SEQ ID NO: 9 - protein, 8 aa, synthetic construct
  REGION 1..8: note = B391-A04 HCDR1
GGTFSSRT

SEQ ID NO: 10 - protein, 8 aa, synthetic construct
  REGION 1..8: note = B391-A04/B391-G06 HCDR2
MTWIGDVG

SEQ ID NO: 11 - protein, 22 aa, synthetic construct
  REGION 1..22: note = B391-A04 HCDR3
GASRGGSYSMVIHTTSPNDYDY

SEQ ID NO: 12 - protein, 25 aa, synthetic construct
  REGION 1..25: note = B391-A04 H-FR1
QVQLVESGGGLVQAGGSLRLSCTAS

SEQ ID NO: 13 - protein, 17 aa, synthetic construct
  REGION 1..17: note = B391-A04 H-FR2
MGWFRQPPGKEREFVAI

SEQ ID NO: 14 - protein, 38 aa, synthetic construct
  REGION 1..38: note = B391-A04/B391-G06 H-FR3
LYADSVKGRFTISRDNARNTLYLQMNNLKPEDTAVYYC

SEQ ID NO: 15 - protein, 11 aa, synthetic construct
  REGION 1..11: note = B391-A04/B391-G06/B393-D07/B39C6-G06/B39C8-G05 H-FR4
WGQGTQVTVSS

SEQ ID NO: 16 - protein, 129 aa, synthetic construct
  REGION 1..129: note = B391-A04 VHH
QVQLVESGGGLVQAGGSLRLSCTASGGTFSSRTMGWFRQPPGKEREFVAIMTWIGDVGLYADSVKGRFTISRDNARNTLYLQMNNLKPEDTAVYYCGASRGGSYSMVIHTTSPNDYDYWGQGTQVTVSS

SEQ ID NO: 17 - protein, 8 aa, synthetic construct
  REGION 1..8: note = B391-G06 HCDR1
GGTFRSKT

SEQ ID NO: 18 - protein, 23 aa, synthetic construct
  REGION 1..23: note = B391-G06 HCDR3
GASRGGPPYSMVVHTTSPNGYDY

SEQ ID NO: 19 - protein, 25 aa, synthetic construct
  REGION 1..25: note = B391-G06 H-FR1
QLQLVESGGGLVQTGGSLRLSCTAS

SEQ ID NO: 20 - protein, 17 aa, synthetic construct
  REGION 1..17: note = B391-G06 H-FR2
MGWFRQAPGKEREFVAI

SEQ ID NO: 21 - protein, 130 aa, synthetic construct
  REGION 1..130: note = B391-G06 VHH
QLQLVESGGGLVQTGGSLRLSCTASGGTFRSKTMGWFRQAPGKEREFVAIMTWIGDVGLYADSVKGRFTISRDNARNTLYLQMNNLKPEDTAVYYCGASRGGPPYSMVVHTTSPNGYDYWGQGTQVTVSS

SEQ ID NO: 22 - protein, 8 aa, synthetic construct
  REGION 1..8: note = B393-D07/B39C6-G06/B39C8-G05 HCDR1
GFTLDYYA

SEQ ID NO: 23 - protein, 8 aa, synthetic construct
  REGION 1..8: note = B393-D07 HCDR2
ISSSNGNI

SEQ ID NO: 24 - protein, 28 aa, synthetic construct
  REGION 1..28: note = B393-D07 HCDR3
AADLSAAPYNDAVRSCTGGSRLRATYDF

SEQ ID NO: 25 - protein, 17 aa, synthetic construct
  REGION 1..17: note = B393-D07 H-FR2
IAWFRQRPGKEREGVSC

SEQ ID NO: 26 - protein, 38 aa, synthetic construct
  REGION 1..38: note = B393-D07 H-FR3
NYADSVKGRFTASRDNAKNTVYLQMNSLKPEDTAVYYC

SEQ ID NO: 27 - protein, 135 aa, synthetic construct
  REGION 1..135: note = B393-D07 VHH
QLQLVESGGGLVQPGGSLRLSCAASGFTLDYYAIAWFRQRPGKEREGVSCISSSNGNINYADSVKGRFTASRDNAKNTVYLQMNSLKPEDTAVYYCAADLSAAPYNDAVRSCTGGSRLRATYDFWGQGTQVTVSS

SEQ ID NO: 28 - protein, 8 aa, synthetic construct
  REGION 1..8: note = B39C6-G06/B39C8-G05 HCDR2
ISSSGGST

SEQ ID NO: 29 - protein, 28 aa, synthetic construct
  REGION 1..28: note = B39C6-G06 HCDR3
AADVSTAPYNDAVRSCTGGNRLASTYDV

SEQ ID NO: 30 - protein, 17 aa, synthetic construct
  REGION 1..17: note = B39C6-G06 H-FR2
IGWFRQAPGKEREGVAC

SEQ ID NO: 31 - protein, 38 aa, synthetic construct
  REGION 1..38: note = B39C6-G06 H-FR3
NYADFVRGRFSSSRDNAKNTVYLQMDSLKPEDTAVYYC

SEQ ID NO: 32 - protein, 135 aa, synthetic construct
  REGION 1..135: note = B39C6-G06 VHH
QLQLVESGGGLVQPGGSLRLSCAASGFTLDYYAIGWFRQAPGKEREGVACISSSGGSTNYADFVRGRFSSSRDNAKNTVYLQMDSLKPEDTAVYYCAADVSTAPYNDAVRSCTGGNRLASTYDVWGQGTQVTVSS

SEQ ID NO: 33 - protein, 28 aa, synthetic construct
  REGION 1..28: note = B39C8-G05 HCDR3
AADLSAAPYNDAVRSCTGGNRLAATYDF

SEQ ID NO: 34 - protein, 25 aa, synthetic construct
  REGION 1..25: note = B39C8-G05 H-FR1
EVQVVESGGGLVQPGGSLRLSCAAS

SEQ ID NO: 35 - protein, 17 aa, synthetic construct
  REGION 1..17: note = B39C8-G05 H-FR2
IAWFRQAPGKGREGVSC

SEQ ID NO: 36 - protein, 38 aa, synthetic construct
  REGION 1..38: note = B39C8-G05 H-FR3
NYADSVKGRFTASRDTAKNTVYLQMNSLKPEDTAVYYC

SEQ ID NO: 37 - protein, 135 aa, synthetic construct
  REGION 1..135: note = B39C8-G05 VHH
EVQVVESGGGLVQPGGSLRLSCAASGFTLDYYAIAWFRQAPGKGREGVSCISSSGGSTNYADSVKGRFTASRDTAKNTVYLQMNSLKPEDTAVYYCAADLSAAPYNDAVRSCTGGNRLAATYDFWGQGTQVTVSS

SEQ ID NO: 38 - protein, 25 aa, synthetic construct [sequence omitted]

SEQ ID NO: 39 - protein, 11 aa, synthetic construct
  REGION 1..11: note = B391-hF04 H-FR4
RGQGTLVTVSS

SEQ ID NO: 40 - protein, 38 aa, synthetic construct
  REGION 1..38: note = B391-hF04 H-FR3
TYQNSVKGRFTISRDNSKNTLYLQMNSLRAEDTAVYYC

SEQ ID NO: 41 - protein, 115 aa, synthetic construct
  REGION 1..115: note = B391-hF04 VHH
EVQLVESGGGLVQPGGSLRLSCAASGFTFSNLGMSWYRQAPGKAREWVGSISASGDYTTYQNSVKGRFTISRDNSKNTLYLQMNSLRAEDTAVYYCTRRVDSYPRGQGTLVTVSS

SEQ ID NO: 42 - protein, 123 aa, synthetic construct
  REGION 1..123: note = H5L5 VH
QVQLVQSGAEVKKPGASVKVSCKASGYNLKDTFLHWVRQAPGQGLEWMGRIDPANGNIKYDPKFQGRVTITADTSANTAYMELISLRSEDTAVYYCANSPYYYGSGYRIFDVWGQGTTVTVSS

SEQ ID NO: 43 - protein, 107 aa, synthetic construct
  REGION 1..107: note = H5L5 VL
QIVLTQSPATLSLSPGERATLSCSAFSSVNYMHWYQQKPGQAPRLLIYTTSNLASGIPTRFSGSGSGTSYTLTISSLEPEDFAVYYCQQRSTYPFTFGQGTKLEIKR

SEQ ID NO: 44 - protein, 229 aa, synthetic construct
  REGION 1..229: note = IgG4Fc
ESKYGPPCPPCPAPEFLGGPSVFLFPPKPKDTLMISRTPEVTCVVVDVSQEDPEVQFNWYVDGVEVHNAKTKPREEQFNSTYRVVSVLTVLHQDWLNGKEYKCKVSNKGLPSSIEKTISKAKGQPREPQVYTLPPSQEEMTKNQVSLTCLVKGFYPSDIAVEWESNGQPENNYKTTPPVLDSDGSFFLYSRLTVDKSRWQEGNVFSCSVMHEALHNHYTQKSLSLSLGK

SEQ ID NO: 45 - protein, 8 aa, synthetic construct
  REGION 1..8: note = YN035 HCDR1
RGPFSTYA

SEQ ID NO: 46 - protein, 8 aa, synthetic construct
  REGION 1..8: note = YN035 HCDR2
IIPILGIA

SEQ ID NO: 47 - protein, 14 aa, synthetic construct
  REGION 1..14: note = YN035 HCDR3
ARTMEGYGFGNFDY

SEQ ID NO: 48 - protein, 121 aa, synthetic construct
  REGION 1..121: note = YN035 VH
QVQLVQSGAEVKKPGSSVKVSCKASRGPFSTYAISWVRQAPGQGLEWMGRIIPILGIANYAQKFQGRVTITADKSTSTAYMELSSLRSEDTAVYYCARTMEGYGFGNFDYWGQGTLVTVSS

SEQ ID NO: 49 - protein, 9 aa, synthetic construct
  REGION 1..9: note = YN035 LCDR1
VSEVGGYNE

SEQ ID NO: 50 - skipped

SEQ ID NO: 51 - protein, 11 aa, synthetic construct
  REGION 1..11: note = YN035 LCDR3
QSYDSSLSGTV

SEQ ID NO: 52 - protein, 112 aa, synthetic construct
  REGION 1..112: note = YN035 VL
QSALTQPASVSGSPGQSITISCTGTVSEVGGYNEVSWYQQHPGKAPKLMIYGNSNRPSGVSNRFSGSKSGNTASLTISGLQAEDEADYYCQSYDSSLSGTVFGGGTKLTVLG

SEQ ID NO: 53 - protein, 8 aa, synthetic construct
  REGION 1..8: note = B391-G06 HCDR1; B391-A04 HCDR1
  SITE 5: note = misc_feature - Xaa = Arg or Ser
  SITE 7: note = misc_feature - Xaa = Lys or Arg
GGTFXSXT

SEQ ID NO: 54 - protein, 23 aa, synthetic construct
  REGION 1..23: note = B391-A04 HCDR3; B391-G06 HCDR3
  SITE 7: note = misc_feature - Xaa = Pro or missing
  SITE 8: note = misc_feature - Xaa = Pro or Ser
  SITE 13: note = misc_feature - Xaa = Ile or Val
  SITE 20: note = misc_feature - Xaa = Asp or Gly
GASRGGXXYSMVXHTTSPNXYDY

SEQ ID NO: 55 - protein, 28 aa, synthetic construct
  REGION 1..28: note = B393-D07 HCDR3; B39C6-G06 HCDR3; B39C8-G05 HCDR3
  SITE 4: note = misc_feature - Xaa = Leu or Val
  SITE 6: note = misc_feature - Xaa = Ala or Thr
  SITE 20: note = misc_feature - Xaa = Asn or Ser
  SITE 23: note = misc_feature - Xaa = Ala or Arg
  SITE 24: note = misc_feature - Xaa = Ala or Ser
  SITE 28: note = misc_feature - Xaa = Phe or Val
AADXSXAPYNDAVRSCTGGXRLXXTYDX

SEQ ID NO: 56 - protein, 25 aa, synthetic construct
  REGION 1..25: note = B391-F04/B393-D07/B39C6-G06 H-FR1; B391-A04 H-FR1; B391-G06 H-FR1; B39C8-G05 H-FR1; B391-hF04 H-FR1
  SITE 1: note = misc_feature - Xaa = Glu or Gln
  SITE 2: note = misc_feature - Xaa = Leu or Val
  SITE 4: note = misc_feature - Xaa = Leu or Val
  SITE 14: note = misc_feature - Xaa = Ala, Pro or Thr
  SITE 23: note = misc_feature - Xaa = Ala or Thr
XXQXVESGGGLVQXGGSLRLSCXAS

SEQ ID NO: 57 - protein, 17 aa, synthetic construct
  REGION 1..17: note = B391-F04/B391-hF04 H-FR2; B391-A04 H-FR2; B391-G06 H-FR2; B39C6-G06 H-FR2; B39C8-G05 H-FR2; B393-D07 H-FR2
  SITE 1: note = misc_feature - Xaa = Ile or Met
  SITE 2: note = misc_feature - Xaa = Ala, Gly or Ser
  SITE 4: note = misc_feature - Xaa = Phe or Tyr
  SITE 7: note = misc_feature - Xaa = Ala, Pro or Arg
  SITE 11: note = misc_feature - Xaa = Ala, Glu or Gly
  SITE 14: note = misc_feature - Xaa = Phe, Gly or Trp
  SITE 16: note = misc_feature - Xaa = Ala, Gly or Ser
  SITE 17: note = misc_feature - Xaa = Cys, Ile or Ser
XXWXRQXPGKXREXVXX

SEQ ID NO: 58 - protein, 38 aa, synthetic construct
  REGION 1..38: note = B391-F04 H-FR3; B391-A04/B391-G06 H-FR3; B393-D07 H-FR3; B39C6-G06 H-FR3; B39C8-G05 H-FR3; B391-hF04 H-FR3
  SITE 1: note = misc_feature - Xaa = Leu, Asn or Thr
  SITE 3: note = misc_feature - Xaa = Ala or Gln
  SITE 4: note = misc_feature - Xaa = Asp or Asn
  SITE 5: note = misc_feature - Xaa = Phe or Ser
  SITE 7: note = misc_feature - Xaa = Lys or Arg
  SITE 11: note = misc_feature - Xaa = Ser or Thr
  SITE 12: note = misc_feature - Xaa = Ala, Ile or Ser
  SITE 16: note = misc_feature - Xaa = Asn or Thr
  SITE 17: note = misc_feature - Xaa = Ala or Ser
  SITE 18: note = misc_feature - Xaa = Lys or Arg
  SITE 21: note = misc_feature - Xaa = Leu or Val
  SITE 26: note = misc_feature - Xaa = Asp or Asn
  SITE 27: note = misc_feature - Xaa = Asn or Ser
  SITE 29: note = misc_feature - Xaa = Lys or Arg
  SITE 30: note = misc_feature - Xaa = Ala or Pro
  SITE 34: note = misc_feature - Xaa = Ala or Gly
XYXXXVXGRFXXSRDXXXNTXYLQMXXLXXEDTXVYYC

SEQ ID NO: 59 - protein, 11 aa, synthetic construct
  REGION 1..11: note = B391-F04 H-FR4; B391-A04/B391-G06/B393-D07/B39C6-G06/B39C8-G05 H-FR4; B391-hF04 H-FR4
  SITE 1: note = misc_feature - Xaa = Arg or Trp
  SITE 6: note = misc_feature - Xaa = Leu or Gln
XGQGTXVTVSS

SEQ ID NO: 60 - protein, 378 aa, synthetic construct
  REGION 1..378: note = MSLN-CART
MALPVTALLLPLALLLHAARPEQKLISEEDLEVQLLESGGGLVQPGGSLRLSCAASGHTDSYYPKAWFRQAPGKEREFVASIGWGGRMTAYADSVKGRFTISRDNSKNTLYLQMNSLRAEDTAVYYCAAGIGWAPTADSGEYDYWGQGTLVTVSSTTTPAPRPPTPAPTIASQPLSLRPEACRPAAGGAVHTRGLDFACDIYIWAPLAGTCGVLLLSLVITLYCKRGRKKLLYIFKQPFMRPVQTTQEEDGCSCRFPEEEEGGCELRVKFSRSADAPAYQQGQNQLYNELNLGRREEYDVLDKRRGRDPEMGGKPRRKNPQEGLYNELQKDKMAEAYSEIGMKGERRRGKGHDGLYQGLSTATKDTYDALHMQALPPR

SEQ ID NO: 61 - protein, 775 aa, synthetic construct
  REGION 1..775: note = MSLN-CART-B391-F04
MALPVTALLLPLALLLHAARPEQKLISEEDLEVQLLESGGGLVQPGGSLRLSCAASGHTDSYYPKAWFRQAPGKEREFVASIGWGGRMTAYADSVKGRFTISRDNSKNTLYLQMNSLRAEDTAVYYCAAGIGWAPTADSGEYDYWGQGTLVTVSSTTTPAPRPPTPAPTIASQPLSLRPEACRPAAGGAVHTRGLDFACDIYIWAPLAGTCGVLLLSLVITLYCKRGRKKLLYIFKQPFMRPVQTTQEEDGCSCRFPEEEEGGCELRVKFSRSADAPAYQQGQNQLYNELNLGRREEYDVLDKRRGRDPEMGGKPRRKNPQEGLYNELQKDKMAEAYSEIGMKGERRRGKGHDGLYQGLSTATKDTYDALHMQALPPRRRKRSGSGEGRGSLLTCGDVEENPGPMDFQVQIFSFLLISASVIISRGAAQPAEVQLVESGGGLVQPGGSLRLSCAASGFTFSNLGMSWYRQAPGKAREWVGSISASGDYTTYQNSVKGRFTISRDNAKNTLYLQMNNLKPEDTGVYYCTRRVDSYPRGQGTQVTVSSESKYGPPCPPCPAPEFLGGPSVFLFPPKPKDTLMISRTPEVTCVVVDVSQEDPEVQFNWYVDGVEVHNAKTKPREEQFNSTYRVVSVLTVLHQDWLNGKEYKCKVSNKGLPSSIEKTISKAKGQPREPQVYTLPPSQEEMTKNQVSLTCLVKGFYPSDIAVEWESNGQPENNYKTTPPVLDSDGSFFLYSRLTVDKSRWQEGNVFSCSVMHEALHNHYTQKSLSLSLGK

SEQ ID NO: 62 - protein, 1140 aa, synthetic construct
  REGION 1..1140: note = MSLN-H5L5
MALPVTALLLPLALLLHAARPEQKLISEEDLEVQLLESGGGLVQPGGSLRLSCAASGHTDSYYPKAWFRQAPGKEREFVASIGWGGRMTAYADSVKGRFTISRDNSKNTLYLQMNSLRAEDTAVYYCAAGIGWAPTADSGEYDYWGQGTLVTVSSTTTPAPRPPTPAPTIASQPLSLRPEACRPAAGGAVHTRGLDFACDIYIWAPLAGTCGVLLLSLVITLYCKRGRKKLLYIFKQPFMRPVQTTQEEDGCSCRFPEEEEGGCELRVKFSRSADAPAYQQGQNQLYNELNLGRREEYDVLDKRRGRDPEMGGKPRRKNPQEGLYNELQKDKMAEAYSEIGMKGERRRGKGHDGLYQGLSTATKDTYDALHMQALPPRRRKRSGSGATNFSLLKQAGDVEENPGPMDFQVQIFSFLLISASVIISRGAAQPAQIVLTQSPATLSLSPGERATLSCSAFSSVNYMHWYQQKPGQAPRLLIYTTSNLASGIPTRFSGSGSGTSYTLTISSLEPEDFAVYYCQQRSTYPFTFGQGTKLEIKRTVAAPSVFIFPPSDEQLKSGTASVVCLLNNFYPREAKVQWKVDNALQSGNSQESVTEQDSKDSTYSLSSTLTLSKADYEKHKVYACEVTHQGLSSPVTKSFNRGECRRKRSGSGEGRGSLLTCGDVEENPGPMGWSCIILFLVATATGVHSQVQLVQSGAEVKKPGASVKVSCKASGYNLKDTFLHWVRQAPGQGLEWMGRIDPANGNIKYDPKFQGRVTITADTSANTAYMELISLRSEDTAVYYCANSPYYYGSGYRIFDVWGQGTTVTVSSASTKGPSVFPLAPCSRSTSESTAALGCLVKDYFPEPVTVSWNSGALTSGVHTFPAVLQSSGLYSLSSVVTVPSSSLGTKTYTCNVDHKPSNTKVDKRVESKYGPPCPPCPAPEFLGGPSVFLFPPKPKDTLMISRTPEVTCVVVDVSQEDPEVQFNWYVDGVEVHNAKTKPREEQFNSTYRVVSVLTVLHQDWLNGKEYKCKVSNKGLPSSIEKTISKAKGQPREPQVYTLPPSQEEMTKNQVSLTCLVKGFYPSDIAVEWESNGQPENNYKTTPPVLDSDGSFFLYSRLTVDKSRWQEGNVFSCSVMHEALHNHYTQKSLSLSLGK

SEQ ID NO: 63 - protein, 759 aa, synthetic construct
  REGION 1..759: note = MSLN-CART-B391-hF04
MALPVTALLLPLALLLHAARPEVQLLESGGGLVQPGGSLRLSCAASGHTDSYYPKAWFRQAPGKEREFVASIGWGGRMTAYADSVKGRFTISRDNSKNTLYLQMNSLRAEDTAVYYCAAGIGWAPTADSGEYDYWGQGTLVTVSSTTTPAPRPPTPAPTIASQPLSLRPEACRPAAGGAVHTRGLDFACDIYIWAPLAGTCGVLLLSLVITLYCKRGRKKLLYIFKQPFMRPVQTTQEEDGCSCRFPEEEEGGCELRVKFSRSADAPAYQQGQNQLYNELNLGRREEYDVLDKRRGRDPEMGGKPRRKNPQEGLYNELQKDKMAEAYSEIGMKGERRRGKGHDGLYQGLSTATKDTYDALHMQALPPRRRKRSGSGEGRGSLLTCGDVEENPGPMETDTLLLWVLLLWVPGSTGDEVQLVESGGGLVQPGGSLRLSCAASGFTFSNLGMSWYRQAPGKAREWVGSISASGDYTTYQNSVKGRFTISRDNSKNTLYLQMNSLRAEDTAVYYCTRRVDSYPRGQGTLVTVSSESKYGPPCPPCPAPEFLGGPSVFLFPPKPKDTLMISRTPEVTCVVVDVSQEDPEVQFNWYVDGVEVHNAKTKPREEQFNSTYRVVSVLTVLHQDWLNGKEYKCKVSNKGLPSSIEKTISKAKGQPREPQVYTLPPSQEEMTKNQVSLTCLVKGFYPSDIAVEWESNGQPENNYKTTPPVLDSDGSFFLYSRLTVDKSRWQEGNVFSCSVMHEALHNHYTQKSLSLSLGK

SEQ ID NO: 64 - protein, 666 aa, synthetic construct
  REGION 1..666: note = MSLN-CART-YN035 (scFv)
MALPVTALLLPLALLLHAARPEVQLLESGGGLVQPGGSLRLSCAASGHTDSYYPKAWFRQAPGKEREFVASIGWGGRMTAYADSVKGRFTISRDNSKNTLYLQMNSLRAEDTAVYYCAAGIGWAPTADSGEYDYWGQGTLVTVSSTTTPAPRPPTPAPTIASQPLSLRPEACRPAAGGAVHTRGLDFACDIYIWAPLAGTCGVLLLSLVITLYCKRGRKKLLYIFKQPFMRPVQTTQEEDGCSCRFPEEEEGGCELRVKFSRSADAPAYQQGQNQLYNELNLGRREEYDVLDKRRGRDPEMGGKPRRKNPQEGLYNELQKDKMAEAYSEIGMKGERRRGKGHDGLYQGLSTATKDTYDALHMQALPPRRRKRSGSGEGRGSLLTCGDVEENPGPMETDTLLLWVLLLWVPGSTGDQVQLVQSGAEVKKPGSSVKVSCKASRGPFSTYAISWVRQAPGQGLEWMGRIIPILGIANYAQKFQGRVTITADKSTSTAYMELSSLRSEDTAVYYCARTMEGYGFGNFDYWGQGTLVTVSSASTGGGGSGGGGSGGGGSQSALTQPASVSGSPGQSITISCTGTVSEVGGYNEVSWYQQHPGKAPKLMIYGNSNRPSGVSNRFSGSKSGNTASLTISGLQAEDEADYYCQSYDSSLSGTVFGGGTKLTVLG

SEQ ID NO: 65 - protein, 1049 aa, synthetic construct
  REGION 1..1049: note = MSLN-CART-B391-hF04-T2A-YN035 (scFv)
MALPVTALLLPLALLLHAARPEVQLLESGGGLVQPGGSLRLSCAASGHTDSYYPKAWFRQAPGKEREFVASIGWGGRMTAYADSVKGRFTISRDNSKNTLYLQMNSLRAEDTAVYYCAAGIGWAPTADSGEYDYWGQGTLVTVSSTTTPAPRPPTPAPTIASQPLSLRPEACRPAAGGAVHTRGLDFACDIYIWAPLAGTCGVLLLSLVITLYCKRGRKKLLYIFKQPFMRPVQTTQEEDGCSCRFPEEEEGGCELRVKFSRSADAPAYQQGQNQLYNELNLGRREEYDVLDKRRGRDPEMGGKPRRKNPQEGLYNELQKDKMAEAYSEIGMKGERRRGKGHDGLYQGLSTATKDTYDALHMQALPPRRRKRSGSGEGRGSLLTCGDVEENPGPMETDTLLLWVLLLWVPGSTGDEVQLVESGGGLVQPGGSLRLSCAASGFTFSNLGMSWYRQAPGKAREWVGSISASGDYTTYQNSVKGRFTISRDNSKNTLYLQMNSLRAEDTAVYYCTRRVDSYPRGQGTLVTVSSESKYGPPCPPCPAPEFLGGPSVFLFPPKPKDTLMISRTPEVTCVVVDVSQEDPEVQFNWYVDGVEVHNAKTKPREEQFNSTYRVVSVLTVLHQDWLNGKEYKCKVSNKGLPSSIEKTISKAKGQPREPQVYTLPPSQEEMTKNQVSLTCLVKGFYPSDIAVEWESNGQPENNYKTTPPVLDSDGSFFLYSRLTVDKSRWQEGNVFSCSVMHEALHNHYTQKSLSLSLGKEGRGSLLTCGDVEENPGPMETDTLLLWVLLLWVPGSTGDQVQLVQSGAEVKKPGSSVKVSCKASRGPFSTYAISWVRQAPGQGLEWMGRIIPILGIANYAQKFQGRVTITADKSTSTAYMELSSLRSEDTAVYYCARTMEGYGFGNFDYWGQGTLVTVSSASTGGGGSGGGGSGGGGSQSALTQPASVSGSPGQSITISCTGTVSEVGGYNEVSWYQQHPGKAPKLMIYGNSNRPSGVSNRFSGSKSGNTASLTISGLQAEDEADYYCQSYDSSLSGTVFGGGTKLTVLG

SEQ ID NO: 66 - protein, 21 aa, synthetic construct
  REGION 1..21: note = CD8 signal peptide
MALPVTALLLPLALLLHAARP

SEQ ID NO: 67 - protein, 124 aa, synthetic construct
  REGION 1..124: note = Anti-MSLN VHH
EVQLLESGGGLVQPGGSLRLSCAASGHTDSYYPKAWFRQAPGKEREFVASIGWGGRMTAYADSVKGRFTISRDNSKNTLYLQMNSLRAEDTAVYYCAAGIGWAPTADSGEYDYWGQGTLVTVSS

SEQ ID NO: 68 - protein, 45 aa, synthetic construct
  REGION 1..45: note = CD8 hinge region
TTTPAPRPPTPAPTIASQPLSLRPEACRPAAGGAVHTRGLDFACD

SEQ ID NO: 69 - protein, 24 aa, synthetic construct
  REGION 1..24: note = CD8 transmembrane domain
IYIWAPLAGTCGVLLLSLVITLYC

SEQ ID NO: 70 - protein, 42 aa, synthetic construct
  REGION 1..42: note = 4-1BB costimulatory domain
KRGRKKLLYIFKQPFMRPVQTTQEEDGCSCRFPEEEEGGCEL

SEQ ID NO: 71 - protein, 112 aa, synthetic construct
  REGION 1..112: note = CD3 zeta
RVKFSRSADAPAYQQGQNQLYNELNLGRREEYDVLDKRRGRDPEMGGKPRRKNPQEGLYNELQKDKMAEAYSEIGMKGERRRGKGHDGLYQGLSTATKDTYDALHMQALPPR